European Patent Specification EP 3 622 089 B1, published July 17, 2024. Title: UNIVERSAL SHORT ADAPTERS FOR INDEXING OF POLYNUCLEOTIDE SAMPLES. Applicant: Illumina, Inc. The sequence listing filed with the application follows.

SEQUENCE LISTING (19 sequences)

SEQ ID NO: 1 - DNA, 19 bp, Artificial Sequence
  Artificial Sequence
agatgtgtataagagacag

SEQ ID NO: 2 - DNA, 19 bp, Artificial Sequence
  Artificial Sequence
ctgtctcttatacacatct

SEQ ID NO: 3 - DNA, 14 bp, Artificial Sequence
  Artificial Sequence
tcgtcggcagcgtc

SEQ ID NO: 4 - DNA, 14 bp, Artificial Sequence
  Artificial Sequence
gacgctgccgacga

SEQ ID NO: 5 - DNA, 15 bp, Artificial Sequence
  Artificial Sequence
gtctcgtgggctcgg

SEQ ID NO: 6 - DNA, 15 bp, Artificial Sequence
  Artificial Sequence
ccgagcccacgagac

SEQ ID NO: 7 - DNA, 24 bp, Artificial Sequence
  Artificial Sequence
caagcagaagacggcatacgagat

SEQ ID NO: 8 - DNA, 29 bp, Artificial Sequence
  Artificial Sequence
aatgatacggcgaccaccgagatctacac

SEQ ID NO: 9 - DNA, 10260 bp, Artificial Sequence
  Artificial Sequence
tgttcaccatcacctgttgcgtaggtggtgacgaacaacaacgccttgttgtattccacctgtaaggtggcacggaacaactcaacgctttctggtatccgagtcataggagactgcgaaagctggaatggatcaaggcatcagtctcgtctgactctaccgaagattcttaggagcctccctctacatgttctcgtgcagcgttggtatataccaacgcaatagctgagggcgatcagacaatataggttggcgcgaacatggttgactgcaaccagtctccattgccgcttgccattaagcgaattaggataggccgagtgcagacagacatgagtgataaccgtaatcggttacggctaccgcctcgcgttattctattcataaggtcctgcggaacaacactgttaggtgtcaccgacatatccaggtgcgcttgatggagtacttcaagacgtccattgcgcggtgccatataaccagtggcacttgacaatgtccgacctaacgtagttcggtagccgcactctattatgtctcagaaccgagtgaggttagacgttaattacgaccggccgtacctcgtgcgtttctacatacacttcaagcggtcctggataaatcaccagcggctgttgatcaatcggctgtggctaatcattaagacaagccggagtggaaacttatcctggtccgcttcctcgcttcggtctatcctaagaacttccttaggtccttcctatggagattcgcaagagccaccacgacatgttgtagtgctcatagattgctgcgagccacagcacggagtgatgtaagaccgttcaaggttacctggaaaagcatcttgggatgctccaaacagacggcggtgagtaatctagtgctcttcgacatctccgtctcatattactctgcgctcagaaggcgctgaggaatagacaccatgtagtgttgcacatgtaacgttgcacggtacctctaggcgcgctcgaatatacaagttattgtggaccgccaatcggcgaaggctaataggaaatgcgaacaggcataggtgtggcctctgtcaattctcacgattctgaatagcctcaggcatgttgttgggcaccaccaaaccaagcagggttggatgaatatcactctgcgctgtctcacgatgcggtttagcataaccgtccaccgctacttgttatcgagaggttcgagagaacctactggcaagagtcaatggagatccgccaattcttattggccactctattgtgtctcgccacatccaggtatgcttgaacgcaagttgacaaggaccagtggttgtatcaggccacgctgaagaatacctataggcgttcgcctaataaccgtcggcggttacgagaggcgttagagaatacccgacagactttagtgagtcattggcttctgccaatcctcaattcttggaggcctccaagtaggctcgcgcgaatctatagttcggagttacctaagaccgcgtgctgtgatacatcacatgtggtccggcacaacttaacagcaatcgttgatggctaccatatgcgattgcgcatagcgcgtccacctatacttgttcgctgacgttgatcagtaccattaaccttcgccggttcctatacgtgaaggcgtacaggaaaggtatggcggaacgcaatatgtctggcctcactcaattcacagtaagatgtgacggagcctgagccggttcagattaactgccggtcagcattaactgaagtactcatggacgtctgcaccgcgtatagttatacgcgagtaacttggtacggtccaaccgcttagaattatccgaggcaacgaggccgggtagaattacctaacacagttcggtgtgatggtagagatcaacgagagcaagcgcgcttggatatatccgtggtatctgacaacgctcaattccataaggccttgcggagctcttaactatctccggtccggatgcttgtaagcatccaaacggtctatggtaactcgcgtggacaagtacaagtggactcctggttgtcttcaaccactcgctatgagctatcgcagacattagtgcgtgccgacataagtagagccggacgagattacgtgcttgcttacatccatcgactgagtagagtcagacgaataatccgtggcggcttacagagaatggttagaggcaacctcacaacagtctgtggtgacgaactgagcgaggtcagataaaggccacggggaattgtaacctgaccactttcagttgtccgcattccgttatgccttacgtattgacgtacgccagtacaaccatagaaggttgcgaggttacgcacctccgtatgttcaagatacacgggagcgtgtaattgatactggccagcgtcacaccgatgtgtgttagcacattggcagcgtccaatgatacgcataagcttatgcggatccgcttctctggatcctctcaacacggctagttgtaatcgactgattatacgcagccgcgtatataacagctcgcggtgatccatagtaaggtgcgacggaagagcgacgatagatagtagcttcttacttgcctccgtccactacacatggtcgtgtgcaaacttacggatgtccgtaagcacagtgtatggtgacacgcattgctctattccatctcgccccaaggccttttggaattcctaatgtgtctcggcacactcactcggcaatgtctaatggcaggatgtgctgaagcacatctatcttgtagcgctccacgattcactcactcctgtctgtcccatcattagttgctgccgaatgagatcatgcagagctgctgtcgctggtcactatcaacctctgcagcgtctcatgataaggataatgtgaagcggcaccgcacgactgtatgtagtcagttaccgtggaccgttacaaaacaagtacaggtggacgtgaacatcgcgcggtgctatattcaccaacttctgttggtccaatggattgaggcaagccagctccactaattcttgtcggcttgttgaatgccaccaggcaacacaggtgggtgtgaacaatccacgtgttcttgtacaccgagcttgccgagatccattacgccatatcttattgcgctcgtaactgaagacggtcaggaaacgcacgagggtatgtagatgccaactggcattggtcaagacgtggtctagtacaactccaacgttcggtggtacctaagcgaactccgataggtcttaatagcggaatgcgataaggctaattagcgtcggccgatacgccacctactattgttcgtccatcgtcatttgctactgcccgtgtcgtggtacactacaaaccgtgtggtgttacacaacgcgtattaatatacgccggctatcggaccgcgctaagttattgaatgttgccaggcaccagaggcctattagaattcgccaattccatctggccttgctctccggactagcttaagtcgatcataccgttctgcgttaccaatctagagaggctcgagagacaactactggtggtcgtcatgtgataactcacagcggtccaataggaattggcgaaggcatggcgcctggcaatattcattaacggtgtccggtaacaccctcacgaggttctgtagaagaattacaagaggccgtggactagattgcgtcgagccataaagacattagggagtgccgaatatgcatgtgcgcatgcacgacgcatcgtagtatgctaccgcagtggcttatgacaatctcactgtccgctgtcacttaaactcgccggggtctattaaaacgttagttggtaccgaccgcgtggatggatacaagcaatggtgttatgcaacaccgcatgtggcgcatcacaatatgcaattggcgccggccaatattacgttagccggtaccgattacctccggttgttcttaaccagagatccgctagagcttatccgaggccaagtagaattggatccgttatgtcttaccgcacaccacagtcggttgtgactattacagttagccgtgaccgacgcagcaatttatgatggccgaagaacgctaggaggtatcccttcgtgatttcctacagcttcctcggtgccttctaacaaggcagctctgaatgatctcgatattgtgtagcgccacacagctaagcgggatcggataactctgtgtattctcacacgcgtaccttccgacgttccttagcaatacattatggcgtgcctgataacgagcagcggtagacgtgtaccagtacacgttgagtaagcaacgacggatggtatgttccggctcaccttaatcttgtctacatccactcgtgcactagatgttgtcgagcaccattaacaagggccggtggaactatagtctttcgcgactccaatattgccaggcgccattgtggccggattcaattaagcctagaactaagcgaggtcggaagcctatgatgattcgcagcatgtgtcaatgcacactggcataagattgggcggagccaatccgtatactcttacgcgtcaatccaattgggcttggccattatgcgtagccgcatacgagcgattggagatagccaagaagtatcagttgacgctgaccctggaactgttcaaggtcaccttgtgtgagtccacacagagatcgtcgcgagctactatactacatgccttcgtgcattcgaagtgaattaggacaggccaaccttatggggttccgcaatcttagctatctccgatcgcagtggttaaggacaaccggagtgctaggttacatcgaacccgtcaccttgtactgttccatgacggccgtcagtaattacttcgccaccgcctattgttaccagtcgacgttgactagtaaaggacgcacggaagtatgtgccatgtgcgattgcacatacagagtccattgagacttgcgaatatgcggaggcgcataacctgcaacctttcatggttcaagttctagtggacctcgaccgtacatacgtacgtgcgtaatacagtgctgcgtgacatcagcgctgtgtgatatcacactcgcaggaagctatgaaggatatgccggtgcgcattaacagtgcattcttacatgcctccgtatggttatacgcaaccgccacacagtattgtgtgacgcagagatagaggagagcgagactcttgcacgtctccatgtaaccagttcaggttgacctgaccggcgatgtttaatagcaccggtaacctgtaacggttcacattcttatgtgcctccgcatctattcagtctcgcctgacgtgcgcgactacatatagtctactactcgtcgtcgtctactggtagttcgcaacgacctagtaacaatctacggtggctcaagccgcaagggattatggagccagcagagattgatgagactctggcgtttctcaataccatcctaatctgcttcggctcccaggcttggttgaatccaacattcacgcttgcctgtatcaaggttgtgaggaaccacagcggaagaaggtaaggaggaagtcgatatcgactagcgctaaccgaaccatgttaggttgctattcaacggcgcctggtaacggtgagacgtaacagagtagcacttgatgatgtccagcacttgattcattccagcctgcaaggtgcggcggaacataatagattaagtggagccggacaacacgttcctgtgtaccttcgtccaagcgtacttggatactatctccaatcgctcttggcgacggtaatgagtaacggcaaagatctctgggagctctcacaggccagcttgaattgatcttgcgtacggccatacgtaagttctacgagacctcgtagacgtgtgtctttacacactccaaccagccacggttgattgtttgtccgctgccacttatcacaacgcgttgtggtataccaccgaatctggttaggctcaacggcagtgtttaatgacaccattatccactgccgcttgtcaagacaagttggagtggacccctgtagagtttcacgagactctcctggcgctcttcaataaaccgagttcggttagacctgccagtcggtattgactaacagaaggacgggaggaagtaaacatcacaatgtgctgtggccacgcgcatgtgtatatgcacggactgtcgtaagtcactatcctattacgcttcgccgtaatgcatatgtgcatgcgcacatatctgcttgcgctcatcctggaggcaatcaagaatggcaccgtcgcctgttactattccgtggaagattacaaggagcgaacggccagaggtaattgagcctaacgtgattcggtacactggttgtagtcaaccacgatctgagtgtgctcagacacatgaggagtgtcagaagacaccgcttgaggttatccagaacatcaccttatgctgttccgcaattggtaggggccaacgaaatgagcggcggcagataataactctcgattgtctctagccagagcgctgggagatatcaatgccacaacgcattgtggtatcgccgtcgtctattactactaattctgctcggcctcatcattaagccatgccggattgccacaccgacgtgtgttagtatcggcacgatctaatgtagcgttcaattggacctggccaacgacgaacagtagtaggtgaaagtgtaacgggacacggtagtcggctcttactaatctccccgatcttatttagctccgccttgagagcttccagagatcgagttaacttagaccggtccaactatgcatggtcgcatgcgaagtcctcgaggacttctatcttatagagctccgcgagagatccgtgtgagcttacacaccaccggagtttgttaagactgaacacctgcaggtgttcaaatagaacgtggcgaggtacctatgttaagtcgcaccggaatcattggatgctgccaagctgcgtcttcgcatactcctaaatctactccggctcgtcttgtgttacagtacaccgtgactcttacgccgctccgtattatagtggcttgcgacaatccataccaaggttcgttggaaccaccggaacgggttaaggtaaccgaagcgctttaggatatctgaagtgcagcaggacatgacaagctcaattggatctggcctcatcctggtctgcttcaacggccttgagtaattccagacctaaggattttcggaagccgttgaggcggaccagaataagagtctgttgagactcaccagttggccaataccaattggctcaccgcgctctgttatatcaggtgcgcaggaacatatgagccgttcttgattacctccaccgcggttctttataacctccgatcgaatttagctaggccaatatgaagcggcgcaggattgacatgaggcagtgcagaagccagaacttattgaggtccgactccttcgagtcttcctactacttagagtcgtccgagattcaagtatgcctggacgcacttacattgttccgtgccacaatgaatacgggcaggcgtacacctctctttgttctctccatgattccgggcagccttaagtatacagagacgcgtgagagttctgtcatacctcactgctgtcgagttgcactagaccaagcggagactgataagagtcgtgatcgcgtacagctatacttaccagatgccgttgagcacaggtataagtgaacgcggagatagccttgagcgattccactggctcgtttcaatctacctacgcgatatcgtatagcgcaaccttcactggttcctgtcgtgtaggacgacacgaagtatcggacgtatctaagtacgcatagtgataggcgacagcgaagttaatgctgaccggcatcagcagcgtgggatgatacaacactctggagtgtctcaagaaagtggtgtaggacaacacgtataggtactcgcgaacgtctcacgtaggtctgtacgaacactgccgcaggtcattatgaaggtggccttgaacaattccttagtcggatccgactaagccatggagcggtgcaagataattgcaacgcgccatggtataacctacaagtgttcgtggactagctcacagcgatctgtgataggtatgttcgaacgcaccgctctgacggatctcagtaaagcacctgcggatgttcatagagccactcgagattgtctactaccatcattcgttgctgccattgtaccttgccacgttcttggcctaggccaattcgaaagtcacgtgtgactgtacacgcttagtcagatccgactgaacgaatagatgtaggcgagcatattaggctgcgccgaatctcagctgcctctgatcattcccaagaggtgttggagaacaaatccgccttggcttattccaactacattgggtcgtgccagtcatgcaatactgcatggccgtaggctgttacgaatcactaaggtcgttcggaactaccaccttccgcggttccttatagcagacacggatgagtgtaacaatccttgttggcttccaccgacaaggattagtggaagcaatgtcggaaggcactaagggctagactatatcgagtcgctgatgcactgcagcatgtcagcttcatattatcctgcgccactatgatcggtcgcagctatagagaccggcgagagttaaagacgatgcggagtagcatagacaattgagagtggccagaccaagtaactttggacggtcgccttcagttattcctgaccagacctacatgagttcgtgctcctcggactcttctaagtcactcaactaggtctggtcgattagaccatgccgagttgcatggttctcatcaacctctgcagtgcgagtggacatagacaatgtgactcggcacagtctacggctgcagttaatcatgactacaagacttcgtggagtcccatatcttcgtgcgctcctaacgagagaaggtagagaggattacttctggccgtcctcaagatactaccgagcgtcgttaaggtgtaggtgaacacgaactggataggatcaagcgaagctatgaacttgcgcaggtccaaatcgcgtcaggctatactgagtccggagggacttaagaaattctcacgtgcctctgtactggtcatggtcaactgcaacgtccgtcctgacttacttcagccgaggagtattagaagactcgacgctagctagtatcgactgaattagttcaggccgaccttggtctcgtccaactctacggtcggcattaactaatgcatataatccggcgcggcttaataaggcagtgcggaatgacaactgtcgtgggtcactacaaggctgaacggaatcaggtaaaggaagagtggaaggagacccttgcctagttccattcgactcaagttcttctggacctcacagaattctgtgaggcctcgctaggaagtatcgaaggacatactctagggcgtctcgaagttccgaacgaccttaggtaaagagagtctggagagactcttcgaagaggcctaggagaaaaggcttcatggaatcctgctctacgaatgctcgtaggcagatcagcactagctgatgtcccgctccgttttatcttaccttgtgtggttccacacaacctaggttacctcgaaccgttcaagcctaataggattcggcgtgtacaatagcacgtggcgaaccgattattgttagccgccaagaggatgaggagaagcagtgttcgatgtcacctagcaccggttaatagtaaccggcgatagcgttgctcgataccatcaccatacctggttgcgttcatgcaatgaatcatggcaggcgcaggaccgtatgaagttactctcgctaagctctatcggattcagcattgcctgatgccacacgtcagagtgtactgagactctcctccttctcttcttcacggattcgggtaagcctaagcgaccgatgatagttagcagaatgtcagtaggcactgacgctcgcacatatctatgtgccagacgtggttgagtacaacacatctgagggtgctcagaaattctagctggcctcgatcaaatgactggtggcagtcaactccttcgaagcttcctaggagactggagctagtcaagatcatgtcgtattgcactacgccaagattcgtaggagcctacggatcgatcctagctagcttcagttcctcgggaccttctaaaggagtcgaggaagactaga

SEQ ID NO: 10 - DNA, 960 bp, Artificial Sequence
  Artificial Sequence
ggatatatccaagcgcgcttcaacgagagctggtagagatttcggtgtgacctaacacagggtagaattaaacgaggccgtatccgaggccgcttagaatacggtccaacgtaacttggtttatacgcgaccgcgtataggacgtctgcaagtactcatgcattaactgatgccggtcagtcagattaacctgagccggtgtgacggagcacagtaagatcactcaattctgtctggcctgaacgcaataaggtatggcgcgtacaggaatacgtgaaggccggttcctattaaccttcgatcagtaccagctgacgttgatacttgttcgcgtccaccttgcgcatagccatatgcgattgatggctaccagcaatcgtcacaacttaatgtggtccggatacatcacagcgtgctgtgacctaagaccgttcggagttcgaatctatataggctcgcgggcctccaagaattcttggagccaatcctcattggcttctttagtgagtcccgacagacttagagaataccgagaggcgttcggcggttactaataaccgaggcgttcgcgaatacctatccacgctgaattgtatcaggggaccagtggaagttgacaagcttgaacgcatccaggtatgtctcgccacactctattgtcttattggcctccgccaatttcaatggagactggcaagagagagaacctagagaggttcgacttgttatcgtccaccgcttagcataacccgatgcggttcgctgtctcatatcactctggttggatgaaaccaagcagggcaccaccaaatgttgttggagcctcaggcgattctgaatcaattctcactggcctctgtggcataggtgaatgcgaacagctaataggaatcggcgaagtggaccgccacaagttattgctcgaatatatctaggcgcggcacggtaccatgtaacgtt

SEQ ID NO: 11 - DNA, 960 bp, Artificial Sequence
  Artificial Sequence
tgttcaccatcacctgttgcgtaggtggtgacgaacaacaacgccttgttgtattccacctgtaaggtggcacggaacaactcaacgctttctggtatccgagtcataggagactgcgaaagctggaatggatcaaggcatcagtctcgtctgactctaccgaagattcttaggagcctccctctacatgttctcgtgcagcgttggtatataccaacgcaatagctgagggcgatcagacaatataggttggcgcgaacatggttgactgcaaccagtctccattgccgcttgccattaagcgaattaggataggccgagtgcagacagacatgagtgataaccgtaatcggttacggctaccgcctcgcgttattctattcataaggtcctgcggaacaacactgttaggtgtcaccgacatatccaggtgcgcttgatggagtacttcaagacgtccattgcgcggtgccatataaccagtggcacttgacaatgtccgacctaacgtagttcggtagccgcactctattatgtctcagaaccgagtgaggttagacgttaattacgaccggccgtacctcgtgcgtttctacatacacttcaagcggtcctggataaatcaccagcggctgttgatcaatcggctgtggctaatcattaagacaagccggagtggaaacttatcctggtccgcttcctcgcttcggtctatcctaagaacttccttaggtccttcctatggagattcgcaagagccaccacgacatgttgtagtgctcatagattgctgcgagccacagcacggagtgatgtaagaccgttcaaggttacctggaaaagcatcttgggatgctccaaacagacggcggtgagtaatctagtgctcttcgacatctccgtctcatattactctgcgctcagaaggcgctgaggaatagacaccatgtagtgttgcac

SEQ ID NO: 12 - DNA, 960 bp, Artificial Sequence
  Artificial Sequence
agtgttgcacgacaccatgtctgaggaatatcagaaggcgtactctgcgccgtctcatattcgacatctcctagtgctctggtgagtaataacagacggcggatgctccaaagcatcttgttacctggaaccgttcaaggtgatgtaagacagcacggagctgcgagccatcatagattggttgtagtgcaccacgacatcgcaagagcctatggagattaggtccttccgaacttcctttctatcctaactcgcttcggggtccgcttcaacttatcctccggagtggattaagacaagtggctaatcacaatcggctgggctgttgataatcaccagcgtcctggataacttcaagcgttctacataccctcgtgcgtaccggccgtagttaattacggaggttagacagaaccgagtattatgtctcgccgcactcttagttcggtacgacctaacgtgacaatgtccagtggcactgccatataacattgcgcggtcaagacgtcctggagtacttgtgcgcttgaacatatccagggtgtcaccgaacactgttacctgcggaacttcataaggtcgttattctataccgcctcgcggttacggctaaccgtaatacatgagtgagtgcagacaggataggccgaagcgaattagcttgccattatccattgccggcaaccagtcatggttgacttggcgcgaaccaatataggtggcgatcagaaatagctgagataccaacgcgcgttggtatttctcgtgcacctctacatgtaggagcctccgaagattctctgactctactcagtctcgtgatcaaggcaagctggaatgagactgcgaagagtcataggtctggtatccctcaacgcttcacggaacaatgtaaggtgggtattccaccacgccttgttacgaacaacagtaggtggtgcacctgttgctgttcaccat

SEQ ID NO: 13 - DNA, 960 bp, Artificial Sequence
  Artificial Sequence
atgtaacgttgcacggtacctctaggcgcgctcgaatatacaagttattgtggaccgccaatcggcgaaggctaataggaaatgcgaacaggcataggtgtggcctctgtcaattctcacgattctgaatagcctcaggcatgttgttgggcaccaccaaaccaagcagggttggatgaatatcactctgcgctgtctcacgatgcggtttagcataaccgtccaccgctacttgttatcgagaggttcgagagaacctactggcaagagtcaatggagatccgccaattcttattggccactctattgtgtctcgccacatccaggtatgcttgaacgcaagttgacaaggaccagtggttgtatcaggccacgctgaagaatacctataggcgttcgcctaataaccgtcggcggttacgagaggcgttagagaatacccgacagactttagtgagtcattggcttctgccaatcctcaattcttggaggcctccaagtaggctcgcgcgaatctatagttcggagttacctaagaccgcgtgctgtgatacatcacatgtggtccggcacaacttaacagcaatcgttgatggctaccatatgcgattgcgcatagcgcgtccacctatacttgttcgctgacgttgatcagtaccattaaccttcgccggttcctatacgtgaaggcgtacaggaaaggtatggcggaacgcaatatgtctggcctcactcaattcacagtaagatgtgacggagcctgagccggttcagattaactgccggtcagcattaactgaagtactcatggacgtctgcaccgcgtatagttatacgcgagtaacttggtacggtccaaccgcttagaattatccgaggcaacgaggccgggtagaattacctaacacagttcggtgtgatggtagagatcaacgagagcaagcgcgcttggatatatcc

SEQ ID NO: 14 - DNA, 960 bp, Artificial Sequence
  Artificial Sequence
ggtaccgaccaacgttagttggtctattaaaactcgccggctgtcacttatcactgtccgtatgacaatccgcagtggctagtatgctacgacgcatcgtgcgcatgcacatatgcatgtggagtgccgaaagacattagtcgagccatactagattgcgaggccgtggagaattacaagttctgtagaacctcacgaggccggtaacacttaacggtgtgcaatattcaatggcgcctgtggcgaaggccaataggaatcacagcggtctgtgataactgtggtcgtcaacaactactgggctcgagagaatctagagactgcgttacctcataccgttcttaagtcgatccggactagggccttgctcaattccatctagaattcgccgaggcctattccaggcaccattgaatgttgcgctaagttatatcggaccgatacgccggcgcgtattaatgttacacaacaccgtgtggttacactacaacgtgtcgtggtgctactgcccatcgtcattattgttcgtcgccacctactcggccgatactaattagcgtgcgataaggcatagcggaatataggtcttagcgaactccgtggtacctaacaacgttcggagtacaactcgacgtggtctcattggtcaatgccaactggggtatgtagaaacgcacgagacggtcaggagtaactgaagtattgcgctccgccatatctagatccattagagcttgccgcttgtacacctccacgtgttgtgtgaacaaacacaggtggccaccaggcattgttgaatgtcttgtcggcctccactaatggcaagccagaatggattgactgttggtcctcaccaacttggtgctatataacatcgcgcggtggacgtgaacaagtacaaccgttacaagttaccgtggtatgtagtcacgcacgactggaagcggcacaggataatgt

SEQ ID NO: 15 - DNA, 960 bp, Artificial Sequence
  Artificial Sequence
gtggtatctgacaacgctcaattccataaggccttgcggagctcttaactatctccggtccggatgcttgtaagcatccaaacggtctatggtaactcgcgtggacaagtacaagtggactcctggttgtcttcaaccactcgctatgagctatcgcagacattagtgcgtgccgacataagtagagccggacgagattacgtgcttgcttacatccatcgactgagtagagtcagacgaataatccgtggcggcttacagagaatggttagaggcaacctcacaacagtctgtggtgacgaactgagcgaggtcagataaaggccacggggaattgtaacctgaccactttcagttgtccgcattccgttatgccttacgtattgacgtacgccagtacaaccatagaaggttgcgaggttacgcacctccgtatgttcaagatacacgggagcgtgtaattgatactggccagcgtcacaccgatgtgtgttagcacattggcagcgtccaatgatacgcataagcttatgcggatccgcttctctggatcctctcaacacggctagttgtaatcgactgattatacgcagccgcgtatataacagctcgcggtgatccatagtaaggtgcgacggaagagcgacgatagatagtagcttcttacttgcctccgtccactacacatggtcgtgtgcaaacttacggatgtccgtaagcacagtgtatggtgacacgcattgctctattccatctcgccccaaggccttttggaattcctaatgtgtctcggcacactcactcggcaatgtctaatggcaggatgtgctgaagcacatctatcttgtagcgctccacgattcactcactcctgtctgtcccatcattagttgctgccgaatgagatcatgcagagctgctgtcgctggtcactatcaacctctgcagcgtctcatgata

SEQ ID NO: 16 - DNA, 960 bp, Artificial Sequence
  Artificial Sequence
tctcatgatactctgcagcgcactatcaactgtcgctggtgcagagctgcatgagatcatttgctgccgaccatcattagcctgtctgtcttcactcactcgctccacgatatcttgtaggaagcacatcaggatgtgctgtctaatggcactcggcaatcggcacactctaatgtgtctttggaattccccaaggccttccatctcgccttgctctattgtgacacgcaacagtgtatggtccgtaagcacttacggattcgtgtgcaactacacatggcctccgtccattcttacttgagatagtagcgagcgacgattgcgacggaacatagtaaggcgcggtgatctataacagctcagccgcgtatgattatacgtgtaatcgaccacggctagtatcctctcaagcttctctggatgcggatccgcataagcttccaatgatacttggcagcgttgttagcacacaccgatgtggccagcgtcaattgatactgggagcgtgtaaagatacacgccgtatgttcttacgcacctggttgcgaggaaccatagaaacgccagtacgtattgacgttatgccttaccgcattccgtttcagttgtccctgaccactggaattgtaaaaggccacggaggtcagatagaactgagcgctgtggtgactcacaacagtagaggcaaccgagaatggttgcggcttacaataatccgtgagtcagacgagactgagtagtacatccatccgtgcttgctgacgagattaagtagagccgtgccgacatacattagtgcgctatcgcagatcgctatgagcttcaaccactcctggttgtacaagtggacgtggacaagtggtaactcgcaacggtctattaagcatccacggatgcttgatctccggtcgctcttaactgccttgcggaattccataagacaacgctcagtggtatctg

SEQ ID NO: 17 - DNA, 960 bp, Artificial Sequence
  Artificial Sequence
aggataatgtgaagcggcaccgcacgactgtatgtagtcagttaccgtggaccgttacaaaacaagtacaggtggacgtgaacatcgcgcggtgctatattcaccaacttctgttggtccaatggattgaggcaagccagctccactaattcttgtcggcttgttgaatgccaccaggcaacacaggtgggtgtgaacaatccacgtgttcttgtacaccgagcttgccgagatccattacgccatatcttattgcgctcgtaactgaagacggtcaggaaacgcacgagggtatgtagatgccaactggcattggtcaagacgtggtctagtacaactccaacgttcggtggtacctaagcgaactccgataggtcttaatagcggaatgcgataaggctaattagcgtcggccgatacgccacctactattgttcgtccatcgtcatttgctactgcccgtgtcgtggtacactacaaaccgtgtggtgttacacaacgcgtattaatatacgccggctatcggaccgcgctaagttattgaatgttgccaggcaccagaggcctattagaattcgccaattccatctggccttgctctccggactagcttaagtcgatcataccgttctgcgttaccaatctagagaggctcgagagacaactactggtggtcgtcatgtgataactcacagcggtccaataggaattggcgaaggcatggcgcctggcaatattcattaacggtgtccggtaacaccctcacgaggttctgtagaagaattacaagaggccgtggactagattgcgtcgagccataaagacattagggagtgccgaatatgcatgtgcgcatgcacgacgcatcgtagtatgctaccgcagtggcttatgacaatctcactgtccgctgtcacttaaactcgccggggtctattaaaacgttagttggtaccgacc

SEQ ID NO: 18 - DNA, 1160 bp, Artificial Sequence
  Artificial Sequence
aggaggtatcgtaccgattatcgcgactcccagcggtagaattgcacataaccacagtcgacatcgaaccataagattggggaagtatgtgcgattggagcgaggtcggattcgccaccgccactcgtgccttgtgtgagtcaaggtcacaggcagctctccttcgtgataaccttatggagctactatatggtgttatgtctcacacgcccgtgaccgaacggatggtacctgcaacctgtaccttccgttatgcgtagcaccttaatccaattaagccaattggcgccgaatatgcggattaacaaggcagagtccatatgtgtcaatcacaatatgcaatccaattgcgaggccaagagcctatgatttcttaaccagcaatacattagtggttaaggagatccgctttgactagtaatacaagcaaaggacaggccctacatgcctcagtaattacactagatgttctccgatcgccttaccgcaccttacgcgtcccttctaacaggcgccattgcgcagcaattgacgctgaccgatcggataacgtcaccttgcgtgtaccagagcgccacacggttccgcaattcctacagccaacaccgcagatcgtcgcgttacagttagctctgtgtatcctattgttatccacacagactggaactgtgaatgatctcttgtctacatccgcatacgatgttccggctggccaatatttggccggattacgttccttagtaagcaacgttcatggttcacgttagccggccatgtgcgctatagtctttgataacgaggaagaacgctgcggagccaaaaggacgcacatagccaagatagaactaaggttgtgactagtgctaggtttccgtatacttccgttatgtgtcgagcacctgacggccgttcttagctatagctaagcgggatattgtgttacacgttgatactgttccaaatattgccattcctcggtgagtatcagtttatgatggcctagaattggatgtggcgcatggcttggccagccggtggaaaggcgcataatgagacttgcgcacactggcgacaaccggaatggcgtgccgcgtggatgggaagtgaatttcgtgcattcagagcttatcccagtcgacgcctccggttggattcgcagc

SEQ ID NO: 19 - DNA, 1160 bp, Artificial Sequence
  Artificial Sequence
aaccttatggaaggacgcacaatattgccaaatccaattgaattggcgccacatcgaaccaccacagtcgacggatggtaacgttagccgacgttccttaactagatgttagagcttatcagcctatgatagcgccacacagctaagcggagctactataaggacaggccaggaggtatcaggcagctctaggcgcataaagtatcagttagtggttaagataagattggatacaagcaaatagccaagaatggcgtgccatgtgtcaatattaacaaggattgcacatacaacaccgcacaattaagcccacaatatgccaccttaatccagagtccatcagcggtagacagtaattacccactcgtgcccagtcgacgccgcatacgaccgtgaccgacctattgttacctccggttgcctgcaacctccttcgtgatccttctaacacgaggccaagcgaggtcggacgcagcaattcgtcaccttgcgtgtaccagctacatgcctctatagtcttctccgatcgcctctgtgtatctggaactgtcttaccgcaccttacgcgtccttgtgtgaggaagaacgctgaagtgaattgaatatgcgggaatgatctcgacaaccggagacgctgaccgagatccgctgatattgtgtgatcggataagatcgtcgcggattcgcagcgcaatacattgcacactggcgccatgtgcggccggtggaagcgattggaggcggagccaagcgtggatggggaagtatgtggccaatattggcgccattgggcttggccaggttccgcaagtaagcaacggtaccgattagtaccttccggtcgagcaccgtgctaggttgttgtgactatacacgttgatactgttccatagaactaagtagaattggatatgatggcctcaaggtcactccacacagatccgtatacttccgttatgttcgcgactcctcgtgcattctctcacacgctcttagctattgacggccgttgagacttgctgataacgagtggccggatttggtgttatgtgtggcgcattgttccggctttacagttagttatgcgtagttcatggttcttcctacagcttcctcggtgttcgccaccgttcttaaccattgactagtattgtctacat